European Patent Specification EP 3 534 945 B1, published April 2, 2025. Title: VACCINE AGAINST PORCINE PARVOVIRUS. Applicant: Boehringer Ingelheim Vetmedica GmbH. The sequence listing filed with the application follows.

SEQUENCE LISTING (16 sequences)

SEQ ID NO: 1 - protein, 579 aa, Porcine parvovirus
MSENVEQHNPINAGTELSATGNESGGGGGGGGGRGAGGVGVSTGSFNNQTEFQYLGEGLVRITAHASRLIHLNMPEHETYKRIHVLNSESGVAGQMVQDDAHTQMVTPWSLIDANAWGVWFNPADWQLISNNMTEINLVSFEQEIFNVVLKTITESATSPPTKIYNNDLTASLMVALDTNNTLPYTPAAPRSETLGFYPWLPTKPTQYRYYLSCTRNLNPPTYTGQSEQITDSIQTGLHSDIMFYTIENAVPIHLLRTGDEFSTGIYHFDTKPLKLTHSWQTNRSLGLPPKLLTEPTTEGDQHPGTLPAANTRKGYHQTINNSYTEATAIRPAQVGYNTPYMNFEYSNGGPFLTPIVPTADTQYNDDEPNGAIRFTMGYQHGQLTTSSQELERYTFNPQSKCGRAPKQQFNQQSPLNLQNTNNGTLLPSDPIGGKTNMHFMNTLNTYGPLTALNNTAPVFPNGQIWDKELDTDLKPRLHVTAPFVCKNNPPGQLFVKIAPNLTDDFNADSPQQPRIITYSNFWWKGTLTFTAKMRSSNMWNPIQQHTTTAENIGNYIPTNIGGIKMFPEYSQLIPRKLY

SEQ ID NO: 2 - protein, 579 aa, Porcine parvovirus
MSENVEQHNPINAGTELSATGNESIGGGGGGGGRGSIGVGVSTGSFNNQTEFQYLGEGLVRITAHASRLIHLNMPEHETYKRIHVLNSESGVAGQMVQDDAHTQMVTPWSLIDANAWGVWFNPADWQLISNNMTEINLVSFEQEIFNVVLKTITESATSPPTKIYNNDLTASLMVALDTNNTLPYTPAAPRSETLGFYPWLPTKPTQYRYYLSCTRNLNPPTYTGQSEQITDSIQTGLHSDIMFYTIENAVPIHLLRTGDEFSTGIYHFDTKPLKLTHSWQTNRSLGLPPKLLTEPTTEGDQHPGTLPAANTRKGYHQTINNSYTEATAIRPAQVGYNTPYMNFEYSNGGPFLTPIVPTADTQYNDDEPNGAIRFTMGYQHGQLTTSSQELERYTFNPQSKCGRAPKQQFNQQSPLNLQNTNNGTLLPSDPIGGKTNMHFMNTLNTYGPLTALNNTAPVFPNGQIWDKELDTDLKPRLHVTAPFVCKNNPPGQLFVKIAPNLTDDFNADSPQQPRIITYSNFWWKGTLTFTAKMRSSNMWNPIQQHTTTAENIGNYIPTNIGGIKMFPEYSQLIPRKLY

SEQ ID NO: 3 - DNA, 1760 bp, Porcine parvovirus
ggatccgccaccatgtccgagaacgtggagcagcacaacccgataaacgcaggcacagagctgtcggcgactggcaatgagagcggaggcggaggcggcggaggaggtggacgcggcgcaggcggagtgggcgtttcgaccggaagcttcaataatcaaaccgagtttcagtacctgggcgagggtttggtgcggattacggctcacgcgtcccgactgatacatctcaatatgccggagcatgagacctacaagcgtatccatgtcctgaactcggaatcgggcgtcgccggtcagatggtccaagatgatgctcatactcagatggtgacaccctggagcttgatagatgccaacgcatggggcgtgtggttcaaccctgcggattggcagctgataagcaataacatgacagaaatcaatttggttagtttcgagcaagagatatttaatgtcgtgctgaaaaccatcacagagagcgccacgagccccccgacgaagatttacaataacgacctgacggcgtccttgatggtcgccttggacacaaataacaccctcccgtacacccccgcggccccccgcagcgagaccctgggcttttatccctggctgcccaccaagccaacgcagtatcgctactacctgagttgtacacgaaatttgaatccgccgacatacactggtcagtcggagcagatcacggacagcattcaaacgggcctgcactccgatatcatgttttacacgatagagaacgcagtacccatccacctgctgcgtacgggagatgagttctcgaccggtatctatcattttgacacaaaacccttgaaattgacgcacagttggcaaaccaatcgctcgctgggcttgcccccaaagttgttgacggaacccaccaccgagggtgaccaacacccaggcactctccccgcagcaaatacccgcaagggctatcatcaaacgatcaacaatagctataccgaggctaccgccattcggccagcacaggtgggatacaacacaccttacatgaactttgaatactccaacggcggcccgttcctgaccccgatagttccgaccgccgacactcagtacaacgatgacgagccgaacggcgccatcaggtttaccatgggctatcagcacggtcaattgacaacttcgtcgcaagaactggaacgctatacattcaaccctcagagtaagtgtggccgggcacccaaacaacagttcaaccagcaatccccactgaacctgcagaataccaacaatggcacgctgctgccatccgatcccattggaggaaagaccaacatgcatttcatgaacacgctgaatacatacggaccactgaccgccctgaacaataccgcacccgtcttccctaatggccagatctgggataaagagctggatacggacctgaagccccgactccacgtgactgcgccctttgtgtgcaaaaataacccaccgggacagttgttcgtcaaaatagcccccaacttgaccgacgacttcaatgcagacagccctcagcagccgcgaatcatcacctattcgaacttctggtggaagggcacgctgactttcacggctaagatgcgctcgagcaatatgtggaacccaatccagcaacataccacaaccgctgaaaatattggcaattacatccctacgaatataggcggaataaagatgtttccggagtattcccagctcattccacgcaagctgtattaagcggccgc

SEQ ID NO: 4 - DNA, 1760 bp, Porcine parvovirus
ggatccgccaccatgtccgagaacgtggagcagcacaacccgataaacgcaggcacagagctgtcggcgactggcaatgaatcgatcggcggaggcggcggaggaggtggacgcggatcgatcggagtgggcgtttcgaccggaagcttcaataatcaaaccgagtttcagtacctgggcgagggtttggtgcggattacggctcacgcgtcccgactgatacatctcaatatgccggagcatgagacctacaagcgtatccatgtcctgaactcggaatcgggcgtcgccggtcagatggtccaagatgatgctcatactcagatggtgacaccctggagcttgatagatgccaacgcatggggcgtgtggttcaaccctgcggattggcagctgataagcaataacatgacagaaatcaatttggttagtttcgagcaagagatatttaatgtcgtgctgaaaaccatcacagagagcgccacgagccccccgacgaagatttacaataacgacctgacggcgtccttgatggtcgccttggacacaaataacaccctcccgtacacccccgcggccccccgcagcgagaccctgggcttttatccctggctgcccaccaagccaacgcagtatcgctactacctgagttgtacacgaaatttgaatccgccgacatacactggtcagtcggagcagatcacggacagcattcaaacgggcctgcactccgatatcatgttttacacgatagagaacgcagtacccatccacctgctgcgtacgggagatgagttctcgaccggtatctatcattttgacacaaaacccttgaaattgacgcacagttggcaaaccaatcgctcgctgggcttgcccccaaagttgttgacggaacccaccaccgagggtgaccaacacccaggcactctccccgcagcaaatacccgcaagggctatcatcaaacgatcaacaatagctataccgaggctaccgccattcggccagcacaggtgggatacaacacaccttacatgaactttgaatactccaacggcggcccgttcctgaccccgatagttccgaccgccgacactcagtacaacgatgacgagccgaacggcgccatcaggtttaccatgggctatcagcacggtcaattgacaacttcgtcgcaagaactggaacgctatacattcaaccctcagagtaagtgtggccgggcacccaaacaacagttcaaccagcaatccccactgaacctgcagaataccaacaatggcacgctgctgccatccgatcccattggaggaaagaccaacatgcatttcatgaacacgctgaatacatacggaccactgaccgccctgaacaataccgcacccgtcttccctaatggccagatctgggataaagagctggatacggacctgaagccccgactccacgtgactgcgccctttgtgtgcaaaaataacccaccgggacagttgttcgtcaaaatagcccccaacttgaccgacgacttcaatgcagacagccctcagcagccgcgaatcatcacctattcgaacttctggtggaagggcacgctgactttcacggctaagatgcgctcgagcaatatgtggaacccaatccagcaacataccacaaccgctgaaaatattggcaattacatccctacgaatataggcggaataaagatgtttccggagtattcccagctcattccacgcaagctgtattaagcggccgc

SEQ ID NO: 5 - protein, 579 aa, Porcine parvovirus
MSENVEQHNPINAGTELSATGNESIGGGGGGGGRGSIGVGVSTGSFNNQTEFQYLGEGLVRITAHASRLIHLNMPEHETYKRIHVLNSESGVAGQMVQDDAHTQMVTPWSLIDANAWGVWFNPADWQLISNNMTEINLVSFEQAIFNVVLKTITESATSPPTKIYNNDLTASLMVALDTNNTLPYTPAAPRSETLGFYPWLPTKPTQYRYYLSCIRNLNPPTYTGQSEQITDSIQTGLHSDIMFYTIENAVPIHLLRTGDEFSTGIYHFDTKPLKLTHSWQTNRSLGLPPKLLTEPTTEGDQHPGTLPAANTRKGYHQTTNNSYTEATAIRPAQVGYNTPYMNFEYSNGGPFLTPIVPTADTQYNDDEPNGAIRFTMDYQHGQLTTSSQELERYTFNPQSKCGRAPKQQFNQQSPLNLQNTNNGTLLPSDPIGGKTNMHFMNTLNTYGPLTALNNTAPVFPNGQIWDKELDTDLKPRLHVTAPFVCKNNPPGQLFVKIAPNLTDDFNADSPQQPRIITYSNFWWKGTLTFTAKMRSSNMWNPIQQHTTTAENIGNYIPTNIGGIRMFPEYSQLIPRKLY

SEQ ID NO: 6 - protein, 579 aa, Porcine parvovirus; identical to SEQ ID NO: 2

SEQ ID NO: 7 - protein, 579 aa, Porcine parvovirus
MSENVEQHNPINAGTELSATGNESIGGGGGGGGRGSIGVGVSTGSFNNQTEFQYLGEGLVRITAHASRLIHLNMPEHETYKRIHVLNSESGVAGQMVQDDAHTQMVTPWSLIDANAWGVWFNPADWQLISNNMTEINLVSFEQEIFNVVLKTITESATSPPTKIYNNDLTASLMVALDTNNTLPYTPAAPRSETLGFYPWLPTKPTQYRYYLSCTRNLNPPTYTGQSEQITDSIQTGLHSDIMFYTIENAVPIHLLRTGDEFSTGIYHFDTKPLKLTHSWQTNRSLGLPPKLLTEPTTEGDQHPGTLPAANTRKGYHQTINNSYTEATAIRPAQVGYNTPYMNFEYSNGGPFFIPIVPTADTQYNDDEPNGGIRFTMGYQHGQLITSSQEVERYTFNPQRKCGRGAKQQFNQQSPLNIQNTNNGTILPSDPIGGKTNMHFMNTPNTYGPLTAVNNTAPVFPNGQIWDKELDTDLKPRLHVTAPFVCKNNPPGQLFVKIAPNLTDDFNADSPQQPRIITYSNFWWKGTLTFTAKMRSSNMWNPIQQHTTTAENIGNYIPTNIGGIKMFPEYSQLIPRKLY

SEQ ID NO: 8 - protein, 579 aa, Porcine parvovirus
MSENVEQHNPINAGTELSATGNESIGGGGGGGGRGSIGVGVSTGSFNNQTEFQYLGEGLVRITAHASRLIHLNMPEHETYKRIHVLNSESGVAGQMVQDDAHTQMVTPWSLIDANAWGVWFNPADWQLISNNMTEINLVSFEQAIFNVVLKTITESATSPPTKIYNNDLTASLMVALHTNNTLPYTPAAPRSETLGFYPWLPTKPTQYRYYLSCIRNLNPPTYTGQSEQITDSIQTGLHSDIMFYTIENAVPIHLLRTGDEFSTGIYHFDTKPLKLTHSWQTNRSLGLPPKLLTEPTTEGDQHPGTLPAANTRKGYHQTINNSYTEATAIRPAQVGYNTPYMNFEYSNGGPFLTPIVPTADTQYNDDEPNGAIRFTMDYQHGHLTTSSQELERYTFNPQSKCGRTPKQQFNQQSPLNLQNTNNGTLLPSDPIGGKTNMHFMNTLNTYGPLTALNNTAPVFPNGQIWDKELDTDLKPRLHVTAPFVCKNNPPGQLFVKIAPNLTDDFNADSPQQPRIITYSNFWWKGTLTFTAKMRSSNMWNPIQQHTTTAENIGKYIPTNIGGIKMFPEYSQLIPRKLY

SEQ ID NO: 9 - protein, 579 aa, Porcine parvovirus
MSENVEQHNPINAGTELSATGNESIGGGGGGGGRGSIGVGVSTGSFNNQTEFQYLGEGLVRITAHASRLIHLNMPEHETYKRIHVLNSESGVAGQMVQDDAHTQMVTPWSLIDANAWGVWFNPADWQLISNNMTEINLVSFEQEIFNVVLKTITESATSPPTKIYNNDLTASLMVALDTNNTLPYTPAAPRSETLGFYPWLPTKPTQYRYYLSCTRNLNPPTYTGQSEQITDSIQTGLHSDIMFYTIENAVPIHLLRTGDEFSTGIYHFDTKPLKLTHSWQTNRSLGLPPKLLTEPTTEGDQHPGTLPAANTRKGYHQTINNSYTEATAIRPAQVGYNTPYMNFEYSNGGPFLTPIVPTADTQYNDDEPNGAIRFTMGYQHGQLTTSSQELERYTFNPQSKCGRAPKQQFNQQSPLNLQNTNNGTLLPSDPIGGKTNMHFMSTLNTYGPLTALNNTAPVFPNGQIWDKELDTDLKPRLHVTAPFVCKNNPPGQLFVKIAPNLTDDFNADSPQQPRIITYSNFWWKGTLTFTAKMRSSNMWNPIQQHTTTAENIGNYIPTNIGGIKMFPEYSQLIPRKLY

SEQ ID NO: 10 - protein, 579 aa, Porcine parvovirus
MSENVEQHNPINAGTELSATGNESIGGGGGGGGRGSIGVGVSTGSFNNQTEFQYLGEGLVRITAHASRLIHLNMPEHETYKRIHVLNSESGVAGQMVQDDAHTQMVTPWSLIDANAWGVWFNPADWQLISNNMTEINLVSFEQEIFNVVLKTITESATSPPTKIYNNDLTASLMVALDTNNTLPYTPAAPRSETLGFYPWLPTKPTQYRYYLSCTRNLNPPTYTGQSEQITDSIQTGLHSDIMFYTIENAVPIHLLRTGDEFSTGIYHFDTKPLKLTHSWQTNRSLGLPPKLLTEPTTEGDQHPGTLPAANTRKGYHQTTNNSYTEATAIRPAQVGYNTPYMNFEYSNGGPFLTPIVPTADTQYNDDEPNGAIRFTMGYQHGQLTTSSQELERYTFNPQSKCGRAPKQQFNQQSPLNLQNTNNGTLLPSDPIGGKTNMHFMNTLNTYGPLTALNNTAPVFPNGQIWDKELDTDLKPRLHVTAPFVCKNNPPGQLFVKIAPNLTDDFNADSPQQPRIITYSNFWWKGTLTFTAKMRSSNMWNPIQQHTTTAENIGNYIPTNIGGIKMFPEYSQLIPRKLY

SEQ ID NO: 11 - protein, 579 aa, Porcine parvovirus
MSENVEQHNPINAGTELSATGNESGGGGGGGGGRGAGGVGVSTGSFNNQTEFQYLGEGLVRITAHASRLIHLNMPEHETYKRIHVLNSESGVAGQMVQDDAHTQMVTPWSLIDANAWGVWFNPADWQLISNNMTEINLVSFEQAIFNVVLKTITESATSPPTKIYNNDLTASLMVALDTNNTLPYTPAAPRSETLGFYPWLPTKPTQYRYYLSCIRNLNPPTYTGQSEQITDSIQTGLHSDIMFYTIENAVPIHLLRTGDEFSTGIYHFDTKPLKLTHSWQTNRSLGLPPKLLTEPTTEGDQHPGTLPAANTRKGYHQTTNNSYTEATAIRPAQVGYNTPYMNFEYSNGGPFLTPIVPTADTQYNDDEPNGAIRFTMDYQHGQLTTSSQELERYTFNPQSKCGRAPKQQFNQQSPLNLQNTNNGTLLPSDPIGGKTNMHFMNTLNTYGPLTALNNTAPVFPNGQIWDKELDTDLKPRLHVTAPFVCKNNPPGQLFVKIAPNLTDDFNADSPQQPRIITYSNFWWKGTLTFTAKMRSSNMWNPIQQHTTTAENIGNYIPTNIGGIRMFPEYSQLIPRKLY

SEQ ID NO: 12 - protein, 579 aa, Porcine parvovirus; identical to SEQ ID NO: 1

SEQ ID NO: 13 - protein, 579 aa, Porcine parvovirus
MSENVEQHNPINAGTELSATGNESGGGGGGGGGRGAGGVGVSTGSFNNQTEFQYLGEGLVRITAHASRLIHLNMPEHETYKRIHVLNSESGVAGQMVQDDAHTQMVTPWSLIDANAWGVWFNPADWQLISNNMTEINLVSFEQEIFNVVLKTITESATSPPTKIYNNDLTASLMVALDTNNTLPYTPAAPRSETLGFYPWLPTKPTQYRYYLSCTRNLNPPTYTGQSEQITDSIQTGLHSDIMFYTIENAVPIHLLRTGDEFSTGIYHFDTKPLKLTHSWQTNRSLGLPPKLLTEPTTEGDQHPGTLPAANTRKGYHQTINNSYTEATAIRPAQVGYNTPYMNFEYSNGGPFFIPIVPTADTQYNDDEPNGGIRFTMGYQHGQLITSSQEVERYTFNPQRKCGRGAKQQFNQQSPLNIQNTNNGTILPSDPIGGKTNMHFMNTPNTYGPLTAVNNTAPVFPNGQIWDKELDTDLKPRLHVTAPFVCKNNPPGQLFVKIAPNLTDDFNADSPQQPRIITYSNFWWKGTLTFTAKMRSSNMWNPIQQHTTTAENIGNYIPTNIGGIKMFPEYSQLIPRKLY

SEQ ID NO: 14 - protein, 579 aa, Porcine parvovirus
MSENVEQHNPINAGTELSATGNESGGGGGGGGGRGAGGVGVSTGSFNNQTEFQYLGEGLVRITAHASRLIHLNMPEHETYKRIHVLNSESGVAGQMVQDDAHTQMVTPWSLIDANAWGVWFNPADWQLISNNMTEINLVSFEQAIFNVVLKTITESATSPPTKIYNNDLTASLMVALHTNNTLPYTPAAPRSETLGFYPWLPTKPTQYRYYLSCIRNLNPPTYTGQSEQITDSIQTGLHSDIMFYTIENAVPIHLLRTGDEFSTGIYHFDTKPLKLTHSWQTNRSLGLPPKLLTEPTTEGDQHPGTLPAANTRKGYHQTINNSYTEATAIRPAQVGYNTPYMNFEYSNGGPFLTPIVPTADTQYNDDEPNGAIRFTMDYQHGHLTTSSQELERYTFNPQSKCGRTPKQQFNQQSPLNLQNTNNGTLLPSDPIGGKTNMHFMNTLNTYGPLTALNNTAPVFPNGQIWDKELDTDLKPRLHVTAPFVCKNNPPGQLFVKIAPNLTDDFNADSPQQPRIITYSNFWWKGTLTFTAKMRSSNMWNPIQQHTTTAENIGKYIPTNIGGIKMFPEYSQLIPRKLY

SEQ ID NO: 15 - protein, 579 aa, Porcine parvovirus
MSENVEQHNPINAGTELSATGNESGGGGGGGGGRGAGGVGVSTGSFNNQTEFQYLGEGLVRITAHASRLIHLNMPEHETYKRIHVLNSESGVAGQMVQDDAHTQMVTPWSLIDANAWGVWFNPADWQLISNNMTEINLVSFEQEIFNVVLKTITESATSPPTKIYNNDLTASLMVALDTNNTLPYTPAAPRSETLGFYPWLPTKPTQYRYYLSCTRNLNPPTYTGQSEQITDSIQTGLHSDIMFYTIENAVPIHLLRTGDEFSTGIYHFDTKPLKLTHSWQTNRSLGLPPKLLTEPTTEGDQHPGTLPAANTRKGYHQTINNSYTEATAIRPAQVGYNTPYMNFEYSNGGPFLTPIVPTADTQYNDDEPNGAIRFTMGYQHGQLTTSSQELERYTFNPQSKCGRAPKQQFNQQSPLNLQNTNNGTLLPSDPIGGKTNMHFMSTLNTYGPLTALNNTAPVFPNGQIWDKELDTDLKPRLHVTAPFVCKNNPPGQLFVKIAPNLTDDFNADSPQQPRIITYSNFWWKGTLTFTAKMRSSNMWNPIQQHTTTAENIGNYIPTNIGGIKMFPEYSQLIPRKLY

SEQ ID NO: 16 - protein, 579 aa, Porcine parvovirus
MSENVEQHNPINAGTELSATGNESGGGGGGGGGRGAGGVGVSTGSFNNQTEFQYLGEGLVRITAHASRLIHLNMPEHETYKRIHVLNSESGVAGQMVQDDAHTQMVTPWSLIDANAWGVWFNPADWQLISNNMTEINLVSFEQEIFNVVLKTITESATSPPTKIYNNDLTASLMVALDTNNTLPYTPAAPRSETLGFYPWLPTKPTQYRYYLSCTRNLNPPTYTGQSEQITDSIQTGLHSDIMFYTIENAVPIHLLRTGDEFSTGIYHFDTKPLKLTHSWQTNRSLGLPPKLLTEPTTEGDQHPGTLPAANTRKGYHQTTNNSYTEATAIRPAQVGYNTPYMNFEYSNGGPFLTPIVPTADTQYNDDEPNGAIRFTMGYQHGQLTTSSQELERYTFNPQSKCGRAPKQQFNQQSPLNLQNTNNGTLLPSDPIGGKTNMHFMNTLNTYGPLTALNNTAPVFPNGQIWDKELDTDLKPRLHVTAPFVCKNNPPGQLFVKIAPNLTDDFNADSPQQPRIITYSNFWWKGTLTFTAKMRSSNMWNPIQQHTTTAENIGNYIPTNIGGIKMFPEYSQLIPRKLY